European Patent Application EP 4 194 557 A1, published June 14, 2023. Title: GENOME EDITING USING CAMPYLOBACTER JEJUNI CRISPR/CAS SYSTEM-DERIVED RGEN. Applicant: TOOLGEN INCORPORATED. Application EP. The sequence listing filed with the application follows.

SEQUENCE LISTING (88 sequences)

SEQ ID NO: 1 - skipped

SEQ ID NO: 2 - RNA, 16 nt, synthetic construct
  misc_feature 1..16: note = stem sequence in guideRNA
  source 1..16: mol_type = other RNA
gttttagtcccttgtg

SEQ ID NO: 3 - skipped

SEQ ID NO: 4 - DNA, 60 bp, homo sapiens
  source 1..60: mol_type = other DNA
cacattaaccggccctgggaatataaggtggtcccagctcggggacacaggatccctgga

SEQ ID NO: 5 - DNA, 58 bp, synthetic construct
  misc_feature 1..58: note = hAAVS1 mutant clone (-2, x1)
  source 1..58: mol_type = other DNA
cacattaaccggccctgggaatataaggtggtcccagcggggacacaggatccctgga

SEQ ID NO: 6 - DNA, 59 bp, synthetic construct
  misc_feature 1..59: note = hAAVS mutant clone (-1, x1)
  source 1..59: mol_type = other DNA
cacattaaccggccctgggaatataaggtggtcccagtcggggacacaggatccctgga

SEQ ID NO: 7 - DNA, 59 bp, mus musculus
  source 1..59: mol_type = other DNA
cttaaaggctaacctggtgtgtgggcgttgtcctgcaggggaattgaacaggtgtaaaa

SEQ ID NO: 8 - DNA, 58 bp, synthetic construct
  misc_feature 1..58: note = Mouse Rosa26 (-1, X1)
  source 1..58: mol_type = other DNA
cttaaaggctaacctggtgtgtgggcttgtcctgcaggggaattgaacaggtgtaaaa

SEQ ID NO: 9 - DNA, 60 bp, synthetic construct
  misc_feature 1..60: note = Mouse Rosa26 (+1, X1)
  source 1..60: mol_type = other DNA
cttaaaggctaacctggtgtgtgggcgtttgtcctgcaggggaattgaacaggtgtaaaa

SEQ ID NO: 10 - DNA, 38 bp, synthetic construct
  misc_feature 1..38: note = Target sequence
  source 1..38: mol_type = other DNA
ggccctgggaatataaggtggtcccagctcggggacac

SEQ ID NO: 11 - DNA, 28 bp, synthetic construct
  misc_feature 1..28: note = GX19
  source 1..28: mol_type = other DNA
gtataaggtggtcccagctcggggacac

SEQ ID NO: 12 - DNA, 29 bp, synthetic construct
  misc_feature 1..29: note = GX20
  source 1..29: mol_type = other DNA
gatataaggtggtcccagctcggggacac

SEQ ID NO: 13 - DNA, 30 bp, synthetic construct
  misc_feature 1..30: note = GX21
  source 1..30: mol_type = other DNA
gaatataaggtggtcccagctcggggacac

SEQ ID NO: 14 - DNA, 31 bp, synthetic construct
  misc_feature 1..31: note = GX22
  source 1..31: mol_type = other DNA
ggaatataaggtggtcccagctcggggacac

SEQ ID NO: 15 - DNA, 32 bp, synthetic construct
  misc_feature 1..32: note = GX23
  source 1..32: mol_type = other DNA
gggaatataaggtggtcccagctcggggacac

SEQ ID NO: 16 - DNA, 30 bp, synthetic construct
  misc_feature 1..30: note = GGX20
  source 1..30: mol_type = other DNA
ggatataaggtggtcccagctcggggacac

SEQ ID NO: 17 - DNA, 31 bp, synthetic construct
  misc_feature 1..31: note = GGGX20
  source 1..31: mol_type = other DNA
gggatataaggtggtcccagctcggggacac

SEQ ID NO: 18 - DNA, 38 bp, synthetic construct; identical to SEQ ID NO: 10
  misc_feature 1..38: note = Target site of hAAVS-CJ1
  source 1..38: mol_type = other DNA

SEQ ID NO: 19 - DNA, 38 bp, synthetic construct
  misc_feature 1..38: note = Target site of hAAVS-NRG1
  source 1..38: mol_type = other DNA
gagaaagggagtagaggcggccacgacctggtgaacac

SEQ ID NO: 20 - DNA, 38 bp, synthetic construct
  misc_feature 1..38: note = Target site of hAAVS-NRG3
  source 1..38: mol_type = other DNA
cgcaccattctcacaaagggagttttccacacggacac

SEQ ID NO: 21 - DNA, 38 bp, synthetic construct
  misc_feature 1..38: note = Target site of hAAVS-NRG5
  source 1..38: mol_type = other DNA
cacctcctgttaggcagattccttatctggtgacacac

SEQ ID NO: 22 - protein, 1003 aa, Campylobacter jejuni
MARILAFDIGISSIGWAFSENDELKDCGVRIFTKVENPKTGESLALPRRLARSARKRLARRKARLNHLKHLIANEFKLNYEDYQSFDESLAKAYKGSLISPYELRFRALNELLSKQDFARVILHIAKRRGYDDIKNSDDKEKGAILKAIKQNEEKLANYQSVGEYLYKEYFQKFKENSKEFTNVRNKKESYERCIAQSFLKDELKLIFKKQREFGFSFSKKFEEEVLSVAFYKRALKDFSHLVGNCSFFTDEKRAPKNSPLAFMFVALTRIINLLNNLKNTEGILYTKDDLNALLNEVLKNGTLTYKQTKKLLGLSDDYEFKGEKGTYFIEFKKYKEFIKALGEHNLSQDDLNEIAKDITLIKDEIKLKKALAKYDLNQNQIDSLSKLEFKDHLNISFKALKLVTPLMLEGKKYDEACNELNLKVAINEDKKDFLPAFNETYYKDEVTNPVVLRAIKEYRKVLNALLKKYGKVHKINIELAREVGKNHSQRAKIEKEQNENYKAKKDAELECEKLGLKINSKNILKLRLFKEQKEFCAYSGEKIKISDLQDEKMLEIDHIYPYSRSFDDSYMNKVLVFTKQNQEKLNQTPFEAFGNDSAKWQKIEVLAKNLPTKKQKRILDKNYKDKEQKNFKDRNLNDTRYIARLVLNYTKDYLDFLPLSDDENTKLNDTQKGSKVHVEAKSGMLTSALRHTWGFSAKDRNNHLHHAIDAVIIAYANNSIVKAFSDFKKEQESNSAELYAKKISELDYKNKRKFFEPFSGFRQKVLDKIDEIFVSKPERKKPSGALHEETFRKEEEFYQSYGGKEGVLKALELGKIRKVNGKIVKNGDMFRVDIFKHKKTNKFYAVPIYTMDFALKVLPNKAVARSKKGEIKDWILMDENYEFCFSLYKDSLILIQTKDMQEPEFVYYNAFTSSTVSLIVSKHDNKFETLSKNQKILFKNANEKEVIAKSIGIQNLKVFEKYIVSALGEVTKAEFRQREDFKKSGPPKKKRKVYPYDVPDYA

SEQ ID NO: 23 - DNA, 100 bp, synthetic construct
  misc_feature 1..100: note = C.jejuni_sgRNA
  misc_feature 1..20: note = n = any nucleotide
  source 1..100: mol_type = other DNA
nnnnnnnnnnnnnnnnnnnngttttagtccctgaaaagggactaaaataaagagtttgcgggactctgcggggttacaatcccctaaaaccgcttttttt

SEQ ID NO: 24 - DNA, 27 bp, synthetic construct
  misc_feature 1..27: note = Target sequence of Human AAVS1
  source 1..27: mol_type = other DNA
atataaggtggtcccagctcggggaca

SEQ ID NO: 25 - DNA, 27 bp, synthetic construct
  misc_feature 1..27: note = Target sequence of Mouse Rosa26
  source 1..27: mol_type = other DNA
attcccctgcaggacaacgcccacaca

SEQ ID NO: 26 - DNA, 20 bp, synthetic construct
  misc_feature 1..20: note = Human AAVS1-F
  source 1..20: mol_type = other DNA
tgcttctcctcttgggaagt

SEQ ID NO: 27 - DNA, 20 bp, synthetic construct
  misc_feature 1..20: note = Human AAVS1-R
  source 1..20: mol_type = other DNA
ccccgttctcctgtggattc

SEQ ID NO: 28 - DNA, 20 bp, synthetic construct
  misc_feature 1..20: note = Mouse Rosa26-F
  source 1..20: mol_type = other DNA
acgtttccgacttgagttgc

SEQ ID NO: 29 - DNA, 20 bp, synthetic construct
  misc_feature 1..20: note = Mouse Rosa26-R
  source 1..20: mol_type = other DNA
cccagctacagcctcgattt

SEQ ID NO: 30 - DNA, 108 bp, synthetic construct
  misc_feature 1..108: note = C.jejuni_sgRNA_stem modified
  misc_feature 1..20: note = n = any nucleotide
  source 1..108: mol_type = other DNA
nnnnnnnnnnnnnnnnnnnngttttagtcccttgtggaaatataagggactaaaataaagagtttgcgggactctgcggggttacaatcccctaaaaccgcttttttt

SEQ ID NO: 31 - DNA, 104 bp, synthetic construct
  misc_feature 1..104: note = C.jejuni_sgRNA_loop modified
  misc_feature 1..20: note = n = any nucleotide
  source 1..104: mol_type = other DNA
nnnnnnnnnnnnnnnnnnnngttttagtccctatattcaaagggactaaaataaagagtttgcgggactctgcggggttacaatcccctaaaaccgcttttttt

SEQ ID NO: 32 - DNA, 27 bp, synthetic construct
  misc_feature 1..27: note = Human AAVS1-CJ1
  source 1..27: mol_type = other DNA
atataaggtggtcccagctcggggaca

SEQ ID NO: 33 - DNA, 27 bp, synthetic construct
  misc_feature 1..27: note = Human AAVS1-NRG1
  source 1..27: mol_type = other DNA
gtagaggcggccacgacctggtgaaca

SEQ ID NO: 34 - DNA, 27 bp, synthetic construct
  misc_feature 1..27: note = Human AAVS1-NRG3
  source 1..27: mol_type = other DNA
tcacaaagggagttttccacacggaca

SEQ ID NO: 35 - DNA, 27 bp, synthetic construct
  misc_feature 1..27: note = Human AAVS1-NRG5
  source 1..27: mol_type = other DNA
taggcagattccttatctggtgacaca

SEQ ID NO: 36 - DNA, 53 bp, synthetic construct
  misc_feature 1..53: note = AS-AV-F1
  source 1..53: mol_type = other DNA
acactctttccctacacgacgctcttccgatctaggaggaggcctaaggatgg

SEQ ID NO: 37 - DNA, 53 bp, synthetic construct
  misc_feature 1..53: note = AS-AV-F2
  source 1..53: mol_type = other DNA
acactctttccctacacgacgctcttccgatctgctctgggcggaggaatatg

SEQ ID NO: 38 - DNA, 53 bp, synthetic construct
  misc_feature 1..53: note = AS-AV-F4
  source 1..53: mol_type = other DNA
acactctttccctacacgacgctcttccgatctatcctctctggctccatcgt

SEQ ID NO: 39 - DNA, 54 bp, synthetic construct
  misc_feature 1..54: note = AS-AV-R1
  source 1..54: mol_type = other DNA
gtgactggagttcagacgtgtgctcttccgatcttgtcatggcatcttccaggg

SEQ ID NO: 40 - DNA, 54 bp, synthetic construct
  misc_feature 1..54: note = AS-AV-R2
  source 1..54: mol_type = other DNA
gtgactggagttcagacgtgtgctcttccgatcttccgtgcgtcagttttacct

SEQ ID NO: 41 - DNA, 54 bp, synthetic construct
  misc_feature 1..54: note = AS-AV-R4
  source 1..54: mol_type = other DNA
gtgactggagttcagacgtgtgctcttccgatctccggttaatgtggctctggt

SEQ ID NO: 42 - DNA, 28 bp, synthetic construct
  misc_feature 1..28: note = Test sequence
  source 1..28: mol_type = other DNA
atataaggtggtcccagctcggggacac

SEQ ID NO: 43 - DNA, 28 bp, synthetic construct
  misc_feature 1..28: note = Test sequence
  source 1..28: mol_type = other DNA
tggccccactgtggggtggaggggacag

SEQ ID NO: 44 - DNA, 28 bp, synthetic construct
  misc_feature 1..28: note = Test sequence
  source 1..28: mol_type = other DNA
caccccacagtggggccactagggacag

SEQ ID NO: 45 - DNA, 28 bp, synthetic construct
  misc_feature 1..28: note = Test sequence
  source 1..28: mol_type = other DNA
ctagcagcaaaccttcccttcactacaa

SEQ ID NO: 46 - DNA, 28 bp, synthetic construct
  misc_feature 1..28: note = Test sequence
  source 1..28: mol_type = other DNA
ctccatgaatgcaaactgttttatacat

SEQ ID NO: 47 - DNA, 28 bp, synthetic construct
  misc_feature 1..28: note = Test sequence
  source 1..28: mol_type = other DNA
tgcattcatggagggcaactaaatacat

SEQ ID NO: 48 - DNA, 28 bp, synthetic construct
  misc_feature 1..28: note = Test sequence
  source 1..28: mol_type = other DNA
atcaagtgtcaagtccaatctatgacat

SEQ ID NO: 49 - DNA, 28 bp, synthetic construct
  misc_feature 1..28: note = Test sequence
  source 1..28: mol_type = other DNA
ccaatctatgacatcaattattatacat

SEQ ID NO: 50 - DNA, 28 bp, synthetic construct
  misc_feature 1..28: note = Test sequence
  source 1..28: mol_type = other DNA
gcaaaaggctgaagagcatgactgacat

SEQ ID NO: 51 - DNA, 28 bp, synthetic construct
  misc_feature 1..28: note = Test sequence
  source 1..28: mol_type = other DNA
gcagcatagtgagcccagaaggggacag

SEQ ID NO: 52 - DNA, 28 bp, synthetic construct
  misc_feature 1..28: note = Test sequence
  source 1..28: mol_type = other DNA
gccgcccagtgggactttggaaatacaa

SEQ ID NO: 53 - DNA, 28 bp, synthetic construct
  misc_feature 1..28: note = Test sequence
  source 1..28: mol_type = other DNA
tccactgcagctcccttactgataacaa

SEQ ID NO: 54 - DNA, 28 bp, synthetic construct
  misc_feature 1..28: note = Test sequence
  source 1..28: mol_type = other DNA
attcccctgcaggacaacgcccacacac

SEQ ID NO: 55 - DNA, 28 bp, synthetic construct
  misc_feature 1..28: note = Test sequence
  source 1..28: mol_type = other DNA
acacctgttcaattcccctgcaggacaa

SEQ ID NO: 56 - DNA, 28 bp, synthetic construct
  misc_feature 1..28: note = Test sequence
  source 1..28: mol_type = other DNA
ttgaacaggtgtaaaattggagggacaa

SEQ ID NO: 57 - DNA, 28 bp, synthetic construct
  misc_feature 1..28: note = Test sequence
  source 1..28: mol_type = other DNA
ttgcccctattaaaaaacttcccgacaa

SEQ ID NO: 58 - DNA, 28 bp, synthetic construct
  misc_feature 1..28: note = Test sequence
  source 1..28: mol_type = other DNA
agatccttactacagtatgaaattacag

SEQ ID NO: 59 - DNA, 28 bp, synthetic construct
  misc_feature 1..28: note = Test sequence
  source 1..28: mol_type = other DNA
agccttatcaaaaggtattttagaacac

SEQ ID NO: 60 - DNA, 28 bp, synthetic construct
  misc_feature 1..28: note = Test sequence
  source 1..28: mol_type = other DNA
cggggcccactcaccgtgcacataacag

SEQ ID NO: 61 - DNA, 28 bp, synthetic construct
  misc_feature 1..28: note = Test sequence
  source 1..28: mol_type = other DNA
gccgtgtccgcgccatggccatctacaa

SEQ ID NO: 62 - DNA, 28 bp, synthetic construct
  misc_feature 1..28: note = Test sequence
  source 1..28: mol_type = other DNA
tggccatctacaagaagtcacagcacat

SEQ ID NO: 63 - DNA, 28 bp, synthetic construct
  misc_feature 1..28: note = Test sequence
  source 1..28: mol_type = other DNA
ccgagtgtcaggagctcctgcagcacag

SEQ ID NO: 64 - DNA, 28 bp, synthetic construct
  misc_feature 1..28: note = Test sequence
  source 1..28: mol_type = other DNA
ctccccggggcccactcaccgtgcacat

SEQ ID NO: 65 - DNA, 28 bp, synthetic construct
  misc_feature 1..28: note = Test sequence
  source 1..28: mol_type = other DNA
cctgtgcagttgtgggtcagcgccacac

SEQ ID NO: 66 - DNA, 28 bp, synthetic construct
  misc_feature 1..28: note = Test sequence
  source 1..28: mol_type = other DNA
ggtgtggcgctgacccacaactgcacag

SEQ ID NO: 67 - DNA, 28 bp, synthetic construct
  misc_feature 1..28: note = Test sequence
  source 1..28: mol_type = other DNA
ttcttgtagatggccatggcgcggacac

SEQ ID NO: 68 - DNA, 28 bp, synthetic construct
  misc_feature 1..28: note = Test sequence
  source 1..28: mol_type = other DNA
cgccatggccatctacaagaagtcacag

SEQ ID NO: 69 - DNA, 28 bp, synthetic construct
  misc_feature 1..28: note = Test sequence
  source 1..28: mol_type = other DNA
acatcatcaatattgttcctgtatacac

SEQ ID NO: 70 - DNA, 28 bp, synthetic construct
  misc_feature 1..28: note = Test sequence
  source 1..28: mol_type = other DNA
tgaatccaaaaaccttaaaacaaaacaa

SEQ ID NO: 71 - DNA, 28 bp, synthetic construct
  misc_feature 1..28: note = Test sequence
  source 1..28: mol_type = other DNA
tgctttgaatccaaaaaccttaaaacaa

SEQ ID NO: 72 - DNA, 28 bp, synthetic construct
  misc_feature 1..28: note = Test sequence
  source 1..28: mol_type = other DNA
agcataaaaaccattacaagatatacaa

SEQ ID NO: 73 - DNA, 28 bp, synthetic construct
  misc_feature 1..28: note = Test sequence
  source 1..28: mol_type = other DNA
gtagatgtgctgagagacattatgacac

SEQ ID NO: 74 - DNA, 28 bp, synthetic construct
  misc_feature 1..28: note = Test sequence
  source 1..28: mol_type = other DNA
ggcggtgtcataatgtctctcagcacat

SEQ ID NO: 75 - DNA, 28 bp, synthetic construct
  misc_feature 1..28: note = Test sequence
  source 1..28: mol_type = other DNA
atttaactgcagaggtatgtataaacat

SEQ ID NO: 76 - DNA, 30 bp, synthetic construct
  misc_feature 1..30: note = Target sequence
  source 1..30: mol_type = other DNA
gccacgacctggtgaacacctaggacgcac

SEQ ID NO: 77 - DNA, 30 bp, synthetic construct
  misc_feature 1..30: note = Target sequence
  source 1..30: mol_type = other DNA
ggccttatctcacaggtaaaactgacgcac

SEQ ID NO: 78 - DNA, 30 bp, synthetic construct
  misc_feature 1..30: note = Target sequence
  source 1..30: mol_type = other DNA
ctcttgggaagtgtaaggaagctgcagcac

SEQ ID NO: 79 - DNA, 30 bp, synthetic construct
  misc_feature 1..30: note = Target sequence
  source 1..30: mol_type = other DNA
agctgcagcaccaggatcagtgaaacgcac

SEQ ID NO: 80 - DNA, 30 bp, synthetic construct
  misc_feature 1..30: note = Target sequence
  source 1..30: mol_type = other DNA
ctgtggggtggaggggacagataaaagtac

SEQ ID NO: 81 - DNA, 30 bp, synthetic construct
  misc_feature 1..30: note = Target sequence
  source 1..30: mol_type = other DNA
gccggttaatgtggctctggttctgggtac

SEQ ID NO: 82 - DNA, 30 bp, synthetic construct
  misc_feature 1..30: note = Target sequence
  source 1..30: mol_type = other DNA
gccatgacagggggctggaagagctagcac

SEQ ID NO: 83 - DNA, 20 bp, synthetic construct
  misc_feature 1..20: note = Target sequence
  source 1..20: mol_type = other DNA
gagaaccagaccacccagaa

SEQ ID NO: 84 - DNA, 20 bp, synthetic construct
  misc_feature 1..20: note = Target sequence
  source 1..20: mol_type = other DNA
ggcagccccgccatcaagaa

SEQ ID NO: 85 - DNA, 20 bp, synthetic construct
  misc_feature 1..20: note = Target sequence
  source 1..20: mol_type = other DNA
gtaagatgcttttctgtgac

SEQ ID NO: 86 - DNA, 20 bp, synthetic construct
  misc_feature 1..20: note = Target sequence
  source 1..20: mol_type = other DNA
gatcctttgatcttttctac

SEQ ID NO: 87 - DNA, 20 bp, synthetic construct
  misc_feature 1..20: note = Target sequence
  source 1..20: mol_type = other DNA
gcctccaaaaaagaagagaa

SEQ ID NO: 88 - DNA, 20 bp, synthetic construct
  misc_feature 1..20: note = Target sequence
  source 1..20: mol_type = other DNA
tgacatcaattattatacat